European Patent Application EP 4 123 028 A2, published January 25, 2023. Title: Nucleic Acid Molecule. Applicant: SUN PHARMACEUTICAL INDUSTRIES AUSTRALIA PTY LIMITED. The sequence listing filed with the application follows.

SEQUENCE LISTING (194 sequences)

SEQ ID NO: 1 - DNA, 2306 bp, Papaver somniferum
cacaccaaacttgatcattgtcataaaaaacagtcctaattgtcatcaatcaaaaacagtcctaacatggctaccaatggcgaaattttcaatacctatggtcataatcatcaatcagccacagtcactaaaatcactgcttctaatgaaagcagcaatggtgtctgttatctttcagaaacggctaacttggggaagttaatatgcattccaatggcactaagagctgcgatggagctaaatgtgttccaacttatctcaaagttcggaactgacgcaaaagtttcggcttctgaaattgcctctaaaatgccaaacgcgaagaataatcctgaagcagctatgtatttggatagaattcttcgactgctcggggcaagttctattctttctgtttctactacaaaaaaatcaatcaacagaggaggagatgatgtagtagtacatgagaagctttatgggttaacaaattcgtcgtgttgtttggtccctcgacaagaagacggggtgtcattagtcgaagaattgctattcacatctgacaaggttgttgtggatagttttttcaaactgaaatgtgtggtggaagaaaaagacagtgtgccatttgaggttgctcatggtgctaaaatctttgagtatgctgctacagaaccaagaatgaatcaagtatttaacgatggaatggcagttttctctattgttgtttttgaggctgtttttagagtttacgatggatttcttgatatgaaagaattgttagatgttggtggtggtattggtacttcggttagtaagattgttgctaaataccctttgattcgcggtgtcaacttcgacttgcctcatgttatttctgttgcccctcaatacccaggtataccttcttcttcttttttctgaaaagaacgggttcgaatttttacagaattttttttctcattcgatactcaagcaactctattaaagtatactgtgtaataatgcatgcaggtgtagagcatgttgcaggagatatgttcgaggaagtcccaaagggtcaaaacatgttgctaaaagtaagctaaccatactcaattttcttaataattaggaaaattgcaaaaaccgtcacaatattataaaggcatctgaagtgccatcactcagataccgatgctatgtactctatacattgacaaaattccatggtatcaagtctcaacctgccggttataataatttttttcaggctttctttaaaagaaattattttgaatggtaaaaatcatcattatattggagaaaagtgcagatcttgctacattaaaatttataatataataaaacatttgtttatggttgtttgaaaaaaaaaatctcattgttaatgcatctttctaagttaatggtgattaatggtgaataatatgatatcttattaccgtcttgacacttttttttttgtcgtagacaaaatatttccaacttttctatattaataaaatcagaaatatttcatttatatgaatattaaaataagaaggtgcatgagtaatattccaaatttcttaaagcgttttttatagcagtacggcgttttctcaaatcttattaacccataattaaagggtttccgtaaattaaattgagggatatcaaaacaaaaacaaaaaatagggttattttgcagtaaaatcaataaccccttatcatatgaaaaggataacttagtctaccccaatttggagagatatgggcaattattgtattactagttcgtttgagcattgataatatttttcattagatttatactcaataaaatatatgaactatattgataaagattaataatgcagtgggtactgcacgattggggtgatgaacgatgtgtgaagctgttaaagaattgttggaactcattacctgtgggtggaaaagttttgataatcgagtttgttctcccgaatgaacttggtaacaatgctgaatcattcaatgcgttgattcccgatttactcctgatggctctgaatccaggcggtaaagagcgaacgatttccgaatacgatgatttaggcaaagcagctggattcataaaaactatacctatccctatctccaatggtcttcatgtcattgagtttcacaaatgaatggttattgagtgctttggtaattaaactaccaagataactacatccatttcatgcatttgctttttttttttcttttttttctttttttttctttttgttttgtattccaggtgtgaactagttagtgtgttgagtggacaaaagtaagtaatcgtattttgtgtt

SEQ ID NO: 2 - DNA, 1440 bp, Papaver somniferum
gaatcagaaactttcttctaaaatctttcaataccagtactgttagtttccgataagagccacactaatccattatggaaattcatttagaaagccaagaacaagaaatgaaatatcaatctcaaatctggaaccaaatatgtggcactgttgatacctctgttctgagatgtgcaattcaattaggtatatttgatgccattcataactctggcaaaccaatgattaccttaaccgaattatcaagcattgtttcatcaccctcttcatcttcaatcgaaccctgcaacttgtatagattagtgagatacttatcccaaatggatctcattagtatcggagaatgtttgaatgaagcaactgtttcattaacaggcacatccaagttactacttagaaaccaagaaaagagtttaattgattgggtattggcaatttcttgcgaaatgatggttgttgtttggcacgaactaagtagctctgtttcaactcctgcggatgagcctccaatcttccagaaggttcatggtaaaaatgctttagaattagcaggggaatttccagaatggaatgatctgatcaacaatgctatgactagtgatactagtgtaactaagccagcgctaatacaaggatgtggcaaaatcctgaacggagttacatcgttaattgatgtcggtggtggtcacggtgccactatggcctacatagttgaagcttttcctcacataaaaggtgcggtaatcgatttaccacatgttgttgaagccgctccggagcgtccaggtgttgagttcatcagcggtgatatattcaagtccatttctaacgctgatgctgtgttgttgaaggtatgtaaagagtagctaaccttagtgcgtctaatttattccacaaatttttctgatgcattttattcttatttttggtttttgcagtatgtcctgcacaattgggaagatacggaatgtgtgaatttactgaagagatgtaaggaagcagttccggcagacaaaggaaaagtgatcataatggatttagtaatagacgacgatgataacagtattttaacgcaggcaaagttgagccttgatctcactgtgatgaaccatggaggaggtagagaaaggactaaagaagattggagaaatctaattgagatgtctggatttagtaggcatgaaataattccaatatctgccatgccatcaattattgttgcttatccttagttaagtcacccgcatgtttacttgaacgggaataagttgggggcgtgttgaatctgttaacatcgcaattgtgcctttactttatgcattctcattccggtagaaactgtttggggcattcggattctgctgagcccttttatgtatgtttgtttgttggttggttggttttcaagtaactgaagtttcttctctgttttcaaggcat

SEQ ID NO: 3 - DNA, 1436 bp, Papaver somniferum
aagttgcaggtagggttatgagcaagctcaattatctctcctataaaagctaacattagaaaaactaataagcacacaaaccgtaaaagttctgaagatagacaaaacaagagaaaaaagatggaagtagtaagtaagattgatcaagaaaaccaagcaaaaatttggaaacaaatttttggttttgcagaatcattagttctaaaatgtgcagttcagttagagattgctgaaacacttcataataatgtaaaacccatgtctttatccgagttagcatctaaacttccggctcaacccgttaatgaagaccgtttgtaccgaattctgcatttcttagttcacatgaaactcttcaacaaagatgctaccacacagaaatattcattagctccaccagcaaagtatttgctaaaaggctgggaaaaatcaatggttccttcaatattaagcgtgactgataaagattttacagctccatggaatcatcttggggacggtttaaccggtaactgtaacgcttttgagaaagcgttaggaaagggcattcgggtttatatgagagaaaatcctgaaaaagatcaattgtttaatgaaggaatggcttgtgatactagattatttgcttcagcattggttaacgagtgcaaaagtattttcagtgacgggatcaatacacttgccggtgttggccgtggtactggtactgcagtgaaagccatatccaaagcttttccggatattaagtgcacaatccatgatcttcctgaagttaccagtaaaaatagtaaaattccaagagatgtttttaagtccgttcctagtgcagacgccatctttatgaaggtaacttctaagaaattttgttttagaatattcgttgcaactctaattgacaacattcataaaaaatatgttaatggtcttaatttattaattctagtagagttacttaaatgatatacaaaaattcaaaatcatataacatttgcagagcattcttcacgaatggaacgatgaggaatgtattcaaatcttgaaacgatgcaaagaagcaataccaaaagggggcaaagttatcattgcggatgtcgtaatagacatggactcgactcatccgtattcaaaatctagactcgcaatggatttggctatgatgctccacacgggtggaaaagagagaactgaagaagattggaaaaaacttattgatgctgcaggttttgctagctgtaaaattactaaactatctgctctccagtctgttattgaggcttaccctcattgaggataatttttatccttctgttttccctttggttaattgttgccttctctttggatcatggttgcgtttataataaatgcagcgtttctttcctggcggtaagtgcaagaaagaaaaagcttccagaaacttccttgagtatgcctgg

SEQ ID NO: 4 - DNA, 1921 bp, Papaver somniferum
cttgagtcatgccttgatatgctcatattttagtttgtcatattcactataactataaatttcaatacaatttctaaaactcatcatcattcaagagagatacaaataccttgatatccttttatcatcaatggagttattcataaagttaccatttatccaaccaattcctttcagtattattcttgttactacagtttcgattgttctattatacagtgtcttcttctgggttactgataagaaaaagaagaggaagaaagcaccaaatgctgcaggggcatggccgttaataggtcatctccgtctattgatgaacgacaaggaaccgttgtatagagcactagggagcatggctgataagtacggacctgcattcaacatccgattaggtaaccaagaagttcttgttgtgagtaactgggagatggtaaaacagtgttttggtaatcaaaatgataagctattttcgaatcgtcaaactacattagctgcaaaatacatgcttaatcaaacaacttctagcggattcgcaccatatggaccatattggagagagctacgaaagataatggtgcagcaattactctctaaacaatctttagaatcgtggaaacatctgaaaatcaaagagatggatgcttcatttagtaaacttaacgagttatgcaacaacaacggtactggaacagctaccctaattaggatggacgaatggtttgctgagttgacgttcaacgtgatcgcaagaaatgtctttggctaccaaagtggcggaaggtcgacagcgcttacgaacggtaatatgatcatactccctcaatctgtatcaatttaaggaaatcattttggtcttgttattaacttgaattttctattaggagatacggaatcaaagggcgagaggtacaagaaaacattggaagaagcacttcatcttatgtcaatttttgcagtttcagacatatttccaagtctagagtgggtagatcggttaagaggccttataaggaatatgaaacgctttggagatgagctaaattcaattgcagggtgtcttattgaagagcaccgccaaaagagattacaatccgtatctaaaagtgataaaggagttggtgatgaacaagacttcgttgatgttctcttatcggttgctgaaaaatcgcaacttcctggagatgaccctgatttggtcatcaagtctatgattctggttaggctattgataccaagtctattgcaattttggtttatgtgcttgttctaactttcgtttactgcatatggatgtgcaggaaatcgtatcaggtgggagtgagaccacatcgtcaaccttaacttgggccctctgtctgttactgaaccatccgcatgtgttaaagaaggcaaaagaggaattagatacgcacgtaggaaaagataggcatgtagaagagtcagatacccctaagctcgtgtacattaatgcaattatcaaagaatcaatgcgattgtatccaaacggggcaatgcttgatcggttggcgttagaagagtgcgaagttggtggatttcatgtaccggccgggggacgcttatttgtcaatgtttggaagattcagagagatccgagtgtttgggagaatcctctggagtttaaaccagagaggtggtttttgagtaatggtgaaaagatggatgtggattacaaaggtcacaatcatgaattcataccatttgggataggtcggaggatgtgcgctggtatgctttgggcatcggaggtgattcatttggtgctgccccgtcttattcatgggtttgatatgaaagcagcaagtgccaatgggaaagtagatatggcagaaatggcaggcatggtgatttgttttaagaagacacctcttgaagttatggtcaatcctcgagagtagatgtt

SEQ ID NO: 5 - DNA, 1688 bp, Papaver somniferum
catgaaattctttatgcaaagagtcaatctgactcaagctagctagaatatataccaatcataaaagaaatgatcatgagtaacttatggattcttacgctcatttctaccatattagcagtctttgctgctgtgttaatcattttcaggagaagaatatcagcatccacaacggaatggcctgttggcccaaaaacattaccaatcataggtaacttgcacattcttggaggcactgctctccatgtcgtcttacataaacttgctgaagtttacggcagtgtaatgacgatatggattggtagttggaaacctgttattattgtttccgactttgatcgagcctgggaagttcttgttaacaaatcgtcagattattcagctcgtgaaatgcctgagatcactaaaatcggcactgcaaattggagaacaatttcaagttctgattctggtccgttttgggccactcttcgaaaaggtcttcagagtgtagcattatcgcctcagcatttagcatcgcaaactgcacaccaagagagagatataataaagttgatcaaaaatttgaaagacgaagcagcttctggaatggttaaaccacttgatcatctcaagaaagcaactgtaagattaatcagtcggttaatctatggtcaggattttgatgacgataagtatgttgaagatatgcatgacgtgatcgagtttttgattcgtattagtggttatgctcaacttgctgaggtattctattatgctaaatatctaccaggtcataagagagctgtaactggcgccgaagaagcaaaaagaagagtaatagctctggtgcgtccttttcttcagtcaaaccctgctactaacacttacttgcattttctcaaatcgcaactgtatcctgaagaggttatcatattcgctatattcgaagcttatcttttaggtgttgatagcacttcttcaaccactgcatgggcactcgcattcttaatacgcgaaccatctgttcaagagaaactttatcaagagcttaagaatttcacagccaataacaatcgcacaatgctgaaagtcgaagacgtcaacaaattaccatatttacaagctgttgttaaagaaacaatgaggatgaaaccaattgcaccactggcgattcctcataaagcttgtaaagacacttcattgatgggcaagaaagttgataagggaactaaagttatggttaacattcatgctttacatcatactgaaaaggtttggaaagaaccttacaaattcataccagagaggtttctgcagaagcacgataaggcgatggaacaatcactattaccatttagtgcaggtatgagaatttgtgcaggaatggaattaggaaaacttcagtttagtttttctcttgctaatcttgttaatgcttttaaatggtcttgtgtgtctgatggagtgcttcctgatatgagtgatttactggggtttgttctgttcatgaaaaccccactcgaagcacgtatagttcctcgtttgtagtgatggaaatttcatctcatgttgttgtttctcttcatgtttactatttcgtactcgtttggttttggtgtaaaaaataagatctaaacttccaaatatcattaatgtttacacaaatcgaaatcaatcaactatgttatgaaaattagtgttttctc

SEQ ID NO: 6 - DNA, 2918 bp, Papaver somniferum
aagtgtgccactaatctactgctagtgctactgctcactgacacttacacatatgattgatttatggctaaacaggatgaccactaaatttattttggaaagcggagtgaattaattaagtggcacattttccatgagaattattgatggcatgcatttagatgaacaagatacaccaaatgtagtgactgaacaagatgctcgatcctaaccccacctgcaactttagctaaactttaataattacatgtcttatctttttattgaatcattttatctatcaatggatgctgatcaataatatcatatatctttgctttttcttcaatcatttagatgaacaaaaaacacaataagtgtagtggttgttcataaccccaccttcaactcattcttccctttaataacaaatatctttgctttttctccaatcatttacttgaacaaccaacactagtaagtgtagtggtttctcataaccccacctgcaatttttgcttacctttaataacatatatctttgattttcttcgatcattttagctaccaatggatgctgatccaaaaagttatggcaaaaagagacaacgtgatcgaacacgagcctctcgtgcaccacagcatcaaggtttgtggaaattaaccgcttgtaaaaaatggagtgcgtgatcataatgaggtattgctaagatatagtatcaactttagtgaactgggccaacaaaactcacgagttgttgaaaattggagattatatttataagataaaagggtcactccctacacaacgacttgcactgcaagtgaaaaagaaaaaaaacaaacaacctcaatctagctagagtcgtgaaaaagttttgtgcgactgttatttagttaattataaaatttcaatgaagtcgttaatgatgaacaagttattatttctccaacggattactgattctccttcgaccaccattatcagtacttttattgttacaataatatccattgtttttctctacactgtcttgttgataaggacgactaagaataagcagaagatagcagcaccaaaagcatcgggggcgtggccgttcataggtcatctcaaactattcatgaaacaagatactcagttttacagaactctaggaaccatgtctgataaatacgggtcggtgttcacacttcgattaggaaaccaagcaatcctagttgtgagcaactgggagatggtaaaagaatgtttcacaacaaacgacaagtcattctcgaatcgtccaagtacgttaagcactaaatacatgctgaatgacactaattctgtcgtgttttcaccttacggaacgtattggagagaaatgcggaagatattggtgcaaaaactactgatctctaaccaaagatcagaggcattgaaaaatctgaaaacgaaagaaatcgacaactcgtttgtaaagcttaatgatttatgcaacaacgatgtcagtggaggaggcacaaaagttaggatggacgaatggttggctgacatgatgttcaacattattgctaggattacatttggttaccaaagcggaggaggcgatgcacctggtatgtgatcatcaaattttcgttaaaaccaaattaacttgtactatatcttatgtttacatgttatattgatcactttgacacgttctgatcattttcacaaatcgaattaggcgcttctacaacatccaagaatgtcgagagatacaagaaaacgttggacgagatgtttgttgttttagcgacgaggtttgcagtttcagatatatttccatctctggagtttatagaccgattgagaggtcttgtaaaggatatgaaaatcttgggagacgaattaaactccattgctggatgttttattgaagaacatcgtcaaaagagacgagaatcattatcctcattgttatctttgtcaaatgaatccgttggtgatgaacaagatttcattgatgttctcttgtcaataatggatcagtcacggcttcccggagatgacccagattttattatcaaaattatgatcctggtaacatatattacaacagtatttctttaagttatggattaatggatgtcgtaaccatgaatatttttctgatctggataaatgtaatccggaactaatatatgaatattgttgacgcaggaagcttttgcaggtgggacggacagtttaagtgcaaccttaacttgggtcctctctctactgctgaaccacccaaacgtgttaaagagggcaagggaggaaatagataggcatgtggaaaacggtaagcaagtggaagtgtctgatattccgaagctcggatacattgatgcaataatcaaagagacgatgagattgtatccagtcggagcattaagcgaacgatacacgactgaagaatgcgaggttggtcggtttaacgtacccgctggcacacgcttactggtgaatatatggaagatccacagagacccaagtgtgtgggagaatccatcagattttcaaccagagaggtttttgtgcagcgataaggtgggtgtggatttatatggccagaattatgagctgataccatttggggccggtaggagggtatgtccggctatagtttcatcactgcagacgatgcattatgcgttggcgcgtcttattcaaggatatgaaatgaaatcagccagcctcgatgggaaggtgaatatggaagaaatgatagccatgtcgtgccacaagatgagccctcttgaagttattatcagtcctcgggagccgaggcggagttaaatcttatgttccaattttacattagcatctttgattatgaaatgtattgctcttaagtttcttttttgttttttatatttttaagcttgtatgtgatcatcagcgaaaatgatgatgacagaatcgt

SEQ ID NO: 7 - DNA, 1915 bp, Papaver somniferum
ttcagttcattcatggcgtatttgatgatcaagaagtctatctatttgttttttgatcaaccaactgcagttggcactcttatacttgcttttctgctgacactttcgcctgttattatttactatgaacagaagaagaggggtttgaggcgaaatcgcaccgcaattacaacgactccattaccagaggcatcaggtgcatggccagtgataggtcatcttcttcttttcatgaacgaaaacgatctaaatcatgtaactcttggtcacatggctgataaatatggacctattttcagcttaagattcggtagacatagaactctagttgttagtagttgggagatggtaaaggagtgttttacaggtaccaatgacaagttgttctcaaatcgtccttcctccttggcggttaaacttatgttttatgacactgaatcttatggttttgcaccttatgggaaatactggagagagttgcgaaagatatctacacacaaactcctctctaatcagcaattagagaagttcaagcacttgcggatttctgaagtcgataactcctttaaaaagcttcatgagttatgcagcaacaacaaacagggaggtgatactacatatgtggctagtcttgtgagaatggatgattggttcgcgtacttgacatttaacgtaataggacggatcgtcagcggattccaatcaaatgcagtggcaggtgagctcatatagctaggtttttatatgtttggtttgtacacacacagctcattcatattctaaactgaattatatgttataattgaacaacataggtgccacaaacagccaggaaaaatacaagcttgcaatcgatgaagtgtcaaatcttatggcaacgtttgccgtttcagatgtggttccacggcttgggtggattgatcgattgactggtcttacaggaaagatgaagaattgtggtaaaaaattagatgcagtagttggggatgcagtggaggatcatcgccaaaagaaactcaaaatttctagaaataacacaggagcacttacggagcacgaagaagaagactttatcgatgtttgcttgtcgattatggagcagtcacagattccgggaaaccaccccgaaatctctgtcaaatctattgccttggtaatacgtctcataagcatgttagcagattttacctctatatatacttacatattattttttatcaatcacacatatgtgcaggacatgttatcgggtgggagtgacactacaaaattgataatgacatggaccctttctttgctgttgaaccatccagacatattggacaaggctaaagaagaagtagatacatacttcgggaagaaaaagatatcggataacacacctgtggttgatgctgccgatgttcctaacctcgtctacatccaagcaatcatcaaagaatcaatgcggttataccctgctagcacattgatggagcgaatgacaagtgatgattgtgatgttggtggcttccacgtaccagctgggacacgattatgggttaacgtatggaagatgcaacgggacccaagggtgtggaaagatccactggtatttctacctgagagattcttgagcaatgacaaagggatggtagatgtgaagggtcagaattatgaactgataccatttggaacaggcaggcggatatgtcctggtgcatcttttgccttggaagtcttgcatttggttcttactcgtcttattcttgagttcgagatgaaggcaccagaggggaaaattgacatgagggcaagaccaggttttttccacaacaaggtggtgccactagatgttcaactcaccccacgcacactagattaagattcctatatatgctaattaattagatgaataaaatctgtggtcgagtaa

SEQ ID NO: 8 - DNA, 1133 bp, Papaver somniferum
aataaaaatccaacaatggcagatccttatgaattcctaatgtgcattcacaatcctgaagaagataccctaacaagaaattttccgattcctgctactcccttagatcaaaacaccaaagacatttctttaaatcctgataggaaaacctcacttcgaatctttcggccaccaaccaaagaacctcctgtaacaaagaataagctgcttcctatcataatttatttccatggtggaggtttcattcttttcaatgcagattcaactatgaaccatgacttttgtcaatcgattgctacacatatacccgcgctggtcgtttctgtagactaccgtcttgctcctgaaaaccgacttcccgctgcctatgatgatgctgttgatgctttaaactgggtcaaagaccaaggtttaggcaaactaaataatagtgaagtatggttaaaagagtatggtgacttctcaaagtgtttcattatggggtgcagctcaggtgctaatgttgcatatcatgccagtttaagagcaatagaaatggatcttgaaccagctaagattaatggattaatattacactgccctttttttggtagtcttgagagaactgaatcagattcaaaagtgatcaacaatcaggacttgccgcttgccgtaagggatgtcatgtgggaactggcgttgccgcttgggtctactcgtgatcacgtttattgtaatccgaatattgatcatgatggatcatcatctggaaatatggtggggttaatcgagagatgttttgtggtaggattttatggggatccacttattgatcgacaaattcagctggtgaagatgctggaggaaaaaggtgtgaaggttgaaacttggattgaacaaggagggtatcatggggtgctatgctttgaccctatgatacgtgaaacctttttggaaaaactaaaacattttattttaaacgacgaatttatatactaaaatatattattagtattaaacaatgaaattcttattttttctaaaatgagcttttggacgaaacattgtgtacgaactagctgatgtaatttttcgttttaccggatttttcattttttttgctttctttctgctctcttttataagtcgttctt

SEQ ID NO: 9 - DNA, 2488 bp, Papaver somniferum
ctaacaggcaaacaataacaggttgcacctacaacattcaatttttattttggtaaatgaagttcagttggagagtaaccacatctttgttgtcggcattgcccccacaatactgagtgttttggctgagtgtagtctgactgtaggtaagctacaactgcatgttgcagataataatcactaactgattattcatgcatacctaacagtcatattgttatagttcccaaaaaaaattctcgaactataaaggcatgcatggacagaaaaatatatcagagagatatcagaaattcaaagagatggaaggaacagggaagatagtatgtgtaacaggtggagctggatacttggcatcttggctgatcatgagattgcttgaacgtggttactctgttcggaccaccgttcggtctgacccaagtacgtaataaattaaatttcctggcatcattttcttcaatataaatttcttattatctagttcatcattctttattgttccaatcatgtccccccaagtctaaaagaagtagtaatctaaaaatagctaatttatgtacgaaattgtaacaatgatctcctagcttatgaggctcacctaatttcgtttctatcattttgtgtcttgaaagaatttagggaagatgtgagccaccttaaagctcttcctgaagctacagagaagcttcaaatttttgaagcagatcttgaaaacccagaaagtttcgacgatgcgatcaacggttgtgtcggtgtctttctcgttgctcaaggaatgaattttgccgaagaatatactcttgaaaaaataatcaaaacatgcgtggaaggaactcttagaattctacagtcatgcttgaaatctaaaacagtgaaaaaggttgtgtacacatcttctgctgatgcagcaatgatgataagtaatctcaaagctgttaaagaaattgacgagacaatatggtcagaagttgacaatttcattagcaaaccggaacaagttattcctggattgccctcatatgtggtttcaaaggtactgacagaaagagcttgcctaaagttttctgaagaacatggtttggatgttgttactatacttcctccgttggttgttggaccttttatcactccccatcctcctcccagtgtatctatagctctttcgataatttcaggtatcctctccatccgaaaaatatgccaattcctaaacttaaaaggcatattgatatttaataatacctccatacctaaaaaaagagttgctatataacatttttaattttcgcccatttttaggcctaattgaaaaagttataataacattttaggaaggagggagaatgatttttgagcaaaccttagaactgtgtggtgagatttgtccgttatcattgttggtataactgtgtatatcatggtttttaaaagcgccgctcacgctacgcttcgtacggttcggtctagatttttttaattcgctccgaagcgtagttatgaagctaccatgaagcgccgcttcacgctacgtttcgtacgcttcgcttcagatttttcaaattcgctccgaggcgaatctaccatgaagtggaagattcctttaattgattcacttttttacttagtcaagtcttttttagggggtttcgaaaactaaagtgaaccactgcgcctcgctactgtttttgaaattaactagacttatattaaattgatacaattattatatcttcctaaatattaaattattaataacaaactactactatttataggaaaaaattcgcttcaaatatcaatcataaaacgacgcttcacatttcaacatgcgcatcgcttcgtataaaaaaaaaacgcttcacgctttcaataccttggtgtacatagattaatacttcctcctctgcgctggtgttaacatttctgtgtttcgtttatatatatgaccaggtgatgtgtcgatgatgcttggtgttagacttgaaaatgcggtacatatagatgatgttgctttagcacacatattcgtttttgaatgtgaaaaagcaaaaggaagacatatttgttcttcagttgattttccaatgcatgatctgcctaaatttatatctgagaattatccggaattcaacgtaccgactgagtgagtttatctttcaccaccttctttattattattcatcaagtcactttgggtattttaaccttattgtttttactgaattatcatcagtttactaaaggatattgaggaacaagaaccagttcatctttcctcagataagctgttgagtatgggatttcagttcaaatatgattttgcagagattttcggtgatgcaatacgatgtgccaaagagaagggtttcctttagagaccaactatagtttggttcggaggagatgtgggagtagctagcccaaaatgccctgctcgcactagcttatattattgttattgtttttcaaatgaataaacgggcag

SEQ ID NO: 10 - DNA, 1572 bp, Papaver somniferum
cgcatataatccaatttgcattgtttatcgaccttgaggaacaattaggggatatggcaacaatgtctagtgctgctgtagaagtgatctcgaaagaaacgattaaaccaagaaatccaacaccatatcaacttagaaactacaatatgtcacttctcgaccaatattcttctctagtttatgttccgatcattcttttctaccctgctgcctccgacgctaatagtaccggaagtaagcaccatgatgatcttcacttgcttaagaggtctctttctgaaacgctagttcacttttatccaatggctggtaggatgaaagacaacatgactgttgactgtaacgacgaaggtattgactttttcgaagtaagaatcaaaggtagaatgtgtgacttcatgatgaaatcagatgcacacttaagtctgcttcttccgtctgaagtcgcttccacgaacttcgtgaaggaagcacaggtgattgttcaagtgaacatgtttgattgcggtggaactgccatttgtttctgtatatcaaacaagattgcagatgcatgcaccatgattaccttcattcgtagtttggcaggcaccaccaacatagctcgtcgtgggagctctattgctgcaccaaccacaaatcagaatttggttccttctttcgattcgacatcactctttccacctagtgaacaattggcatctcaagtttcctatcctacacaggatagtaccagcgtagataaacttgtcagcaaaagatttgtgtttgatgcggcaaagattacatctgcacgtgaaaaattgcaatccttgatgcatgataaatacaaatgccataggccgacaagggttgaggtagtttccgctttgatatggaagtcagcagtgaaatctgctccgcccggttctatatccactgtaacccatgccatgaactttagaaagaaaatggatccaccattacaagatgcgtcattcgggaatctttgtgtggttgttacagcagtattaccagcaacaacggcgacaacaacaaatccagcaaccaaaaaagttagtagtacgagtaatgaagagcaagtggcacttgatgagttaagtgattttgtagccctattgaggcgcgaaatagataaggtaaagggtgataaaggttgcatggagaaaatcattcaaaagttcatctatggtcatgatgcttccgtagcgaaagacagtgatgttgaagataaggtgacagctttgtttatgactagctggtgcaagtttggattctacgaagctgattttggttggggaacgccagtttgggtaactactgttccattaattgagccaaagtacaagaacatggttttcatgaacgatatgaaatgtggtgaaggaattgaagtgtgggtgaattttctggaggatgatatgaccaagttcgaacaccacctaagagagatcctccaactgttttgattttcaaccgtttccctaatagaggtcaattgtcgtgtttgtccatcttaactaccatctttattctcttgttttcatacttgtatttgtcttactccggtaa

SEQ ID NO: 11 - protein, 390 aa, Papaver somniferum
MATNGEIFNTYGHNHQSATVTKITASNESSNGVCYLSETANLGKLICIPMALRAAMELNVFQLISKFGTDAKVSASEIASKMPNAKNNPEAAMYLDRILRLLGASSILSVSTTKKSINRGGDDVVVHEKLYGLTNSSCCLVPRQEDGVSLVEELLFTSDKVVVDSFFKLKCVVEEKDSVPFEVAHGAKIFEYAATEPRMNQVFNDGMAVFSIVVFEAVFRVYDGFLDMKELLDVGGGIGTSVSKIVAKYPLIRGVNFDLPHVISVAPQYPGVEHVAGDMFEEVPKGQNMLLKWVLHDWGDERCVKLLKNCWNSLPVGGKVLIIEFVLPNELGNNAESFNALIPDLLLMALNPGGKERTISEYDDLGKAAGFIKTIPIPISNGLHVIEFHK

SEQ ID NO: 12 - protein, 356 aa, Papaver somniferum
MEIHLESQEQEMKYQSQIWNQICGTVDTSVLRCAIQLGIFDAIHNSGKPMITLTELSSIVSSPSSSSIEPCNLYRLVRYLSQMDLISIGECLNEATVSLTGTSKLLLRNQEKSLIDWVLAISCEMMVVVWHELSSSVSTPADEPPIFQKVHGKNALELAGEFPEWNDLINNAMTSDTSVTKPALIQGCGKILNGVTSLIDVGGGHGATMAYIVEAFPHIKGAVIDLPHVVEAAPERPGVEFISGDIFKSISNADAVLLKYVLHNWEDTECVNLLKRCKEAVPADKGKVIIMDLVIDDDDNSILTQAKLSLDLTVMNHGGGRERTKEDWRNLIEMSGFSRHEIIPISAMPSIIVAYP

SEQ ID NO: 13 - protein, 339 aa, Papaver somniferum
MEVVSKIDQENQAKIWKQIFGFAESLVLKCAVQLEIAETLHNNVKPMSLSELASKLPAQPVNEDRLYRILHFLVHMKLFNKDATTQKYSLAPPAKYLLKGWEKSMVPSILSVTDKDFTAPWNHLGDGLTGNCNAFEKALGKGIRVYMRENPEKDQLFNEGMACDTRLFASALVNECKSIFSDGINTLAGVGRGTGTAVKAISKAFPDIKCTIHDLPEVTSKNSKIPRDVFKSVPSADAIFMKSILHEWNDEECIQILKRCKEAIPKGGKVIIADVVIDMDSTHPYSKSRLAMDLAMMLHTGGKERTEEDWKKLIDAAGFASCKITKLSALQSVIEAYPH

SEQ ID NO: 14 - protein, 540 aa, Papaver somniferum
MELFIKLPFIQPIPFSIILVTTVSIVLLYSVFFWVTDKKKKRKKAPNAAGAWPLIGHLRLLMNDKEPLYRALGSMADKYGPAFNIRLGNQEVLVVSNWEMVKQCFGNQNDKLFSNRQTTLAAKYMLNQTTSSGFAPYGPYWRELRKIMVQQLLSKQSLESWKHLKIKEMDASFSKLNELCNNNGTGTATLIRMDEWFAELTFNVIARNVFGYQSGGRSTALTNGDTESKGERYKKTLEEALHLMSIFAVSDIFPSLEWVDRLRGLIRNMKRFGDELNSIAGCLIEEHRQKRLQSVSKSDKGVGDEQDFVDVLLSVAEKSQLPGDDPDLVIKSMILEIVSGGSETTSSTLTWALCLLLNHPHVLKKAKEELDTHVGKDRHVEESDTPKLVYINAIIKESMRLYPNGAMLDRLALEECEVGGFHVPAGGRLFVNVWKIQRDPSVWENPLEFKPERWFLSNGEKMDVDYKGHNHEFIPFGIGRRMCAGMLWASEVIHLVLPRLIHGFDMKAASANGKVDMAEMAGMVICFKKTPLEVMVNPRE

SEQ ID NO: 15 - protein, 486 aa, Papaver somniferum
MIMSNLWILTLISTILAVFAAVLIIFRRRISASTTEWPVGPKTLPIIGNLHILGGTALHVVLHKLAEVYGSVMTIWIGSWKPVIIVSDFDRAWEVLVNKSSDYSAREMPEITKIGTANWRTISSSDSGPFWATLRKGLQSVALSPQHLASQTAHQERDIIKLIKNLKDEAASGMVKPLDHLKKATVRLISRLIYGQDFDDDKYVEDMHDVIEFLIRISGYAQLAEVFYYAKYLPGHKRAVTGAEEAKRRVIALVRPFLQSNPATNTYLHFLKSQLYPEEVIIFAIFEAYLLGVDSTSSTTAWALAFLIREPSVQEKLYQELKNFTANNNRTMLKVEDVNKLPYLQAVVKETMRMKPIAPLAIPHKACKDTSLMGKKVDKGTKVMVNIHALHHTEKVWKEPYKFIPERFLQKHDKAMEQSLLPFSAGMRICAGMELGKLQFSFSLANLVNAFKWSCVSDGVLPDMSDLLGFVLFMKTPLEARIVPRL

SEQ ID NO: 16 - protein, 554 aa, Papaver somniferum
MKSLMMNKLLFLQRITDSPSTTIISTFIVTIISIVFLYTVLLIRTTKNKQKIAAPKASGAWPFIGHLKLFMKQDTQFYRTLGTMSDKYGSVFTLRLGNQAILVVSNWEMVKECFTTNDKSFSNRPSTLSTKYMLNDTNSVVFSPYGTYWREMRKILVQKLLISNQRSEALKNLKTKEIDNSFVKLNDLCNNDVSGGGTKVRMDEWLADMMFNIIARITFGYQSGGGDAPGASTTSKNVERYKKTLDEMFVVLATRFAVSDIFPSLEFIDRLRGLVKDMKILGDELNSIAGCFIEEHRQKRRESLSSLLSLSNESVGDEQDFIDVLLSIMDQSRLPGDDPDFIIKIMILEAFAGGTDSLSATLTWVLSLLLNHPNVLKRAREEIDRHVENGKQVEVSDIPKLGYIDAIIKETMRLYPVGALSERYTTEECEVGRFNVPAGTRLLVNIWKIHRDPSVWENPSDFQPERFLCSDKVGVDLYGQNYELIPFGAGRRVCPAIVSSLQTMHYALARLIQGYEMKSASLDGKVNMEEMIAMSCHKMSPLEVIISPREPRRS

SEQ ID NO: 17 - protein, 556 aa, Papaver somniferum
MAYLMIKKSIYLFFDQPTAVGTLILAFLLTLSPVIIYYEQKKRGLRRNRTAITTTPLPEASGAWPVIGHLLLFMNENDLNHVTLGHMADKYGPIFSLRFGRHRTLVVSSWEMVKECFTGTNDKLFSNRPSSLAVKLMFYDTESYGFAPYGKYWRELRKISTHKLLSNQQLEKFKHLRISEVDNSFKKLHELCSNNKQGGDTTYVASLVRMDDWFAYLTFNVIGRIVSGFQSNAVAGATNSQEKYKLAIDEVSNLMATFAVSDVVPRLGWIDRLTGLTGKMKNCGKKLDAVVGDAVEDHRQKKLKISRNNTGALTEHEEEDFIDVCLSIMEQSQIPGNHPEISVKSIALDMLSGGSDTTKLIMTWTLSLLLNHPDILDKAKEEVDTYFGKKKISDNTPVVDAADVPNLVYIQAIIKESMRLYPASTLMERMTSDDCDVGGFHVPAGTRLWVNVWKMQRDPRVWKDPLVFLPERFLSNDKGMVDVKGQNYELIPFGTGRRICPGASFALEVLHLVLTRLILEFEMKAPEGKIDMRARPGFFHNKVVPLDVQLTPRTLD

SEQ ID NO: 18 - protein, 320 aa, Papaver somniferum
MADPYEFLMCIHNPEEDTLTRNFPIPATPLDQNTKDISLNPDRKTSLRIFRPPTKEPPVTKNKLLPIIIYFHGGGFILFNADSTMNHDFCQSIATHIPALVVSVDYRLAPENRLPAAYDDAVDALNWVKDQGLGKLNNSEVWLKEYGDFSKCFIMGCSSGANVAYHASLRAIEMDLEPAKINGLILHCPFFGSLERTESDSKVINNQDLPLAVRDVMWELALPLGSTRDHVYCNPNIDHDGSSSGNMVGLIERCFVVGFYGDPLIDRQIQLVKMLEEKGVKVETWIEQGGYHGVLCFDPMIRETFLEKLKHFILNDEFIY

SEQ ID NO: 19 - protein, 348 aa, Papaver somniferum
MHGQKNISERYQKFKEMEGTGKIVCVTGGAGYLASWLIMRLLERGYSVRTTVRSDPKFREDVSHLKALPEATEKLQIFEADLENPESFDDAINGCVGVFLVAQGMNFAEEYTLEKIIKTCVEGTLRILQSCLKSKTVKKVVYTSSADAAMMISNLKAVKEIDETIWSEVDNFISKPEQVIPGLPSYVVSKVLTERACLKFSEEHGLDVVTILPPLVVGPFITPHPPPSVSIALSIISGDVSMMLGVRLENAVHIDDVALAHIFVFECEKAKGRHICSSVDFPMHDLPKFISENYPEFNVPTDLLKDIEEQEPVHLSSDKLLSMGFQFKYDFAEIFGDAIRCAKEKGFL

SEQ ID NO: 20 - protein, 471 aa, Papaver somniferum
MATMSSAAVEVISKETIKPRNPTPYQLRNYNMSLLDQYSSLVYVPIILFYPAASDANSTGSKHHDDLHLLKRSLSETLVHFYPMAGRMKDNMTVDCNDEGIDFFEVRIKGRMCDFMMKSDAHLSLLLPSEVASTNFVKEAQVIVQVNMFDCGGTAICFCISNKIADACTMITFIRSLAGTTNIARRGSSIAAPTTNQNLVPSFDSTSLFPPSEQLASQVSYPTQDSTSVDKLVSKRFVFDAAKITSAREKLQSLMHDKYKCHRPTRVEVVSALIWKSAVKSAPPGSISTVTHAMNFRKKMDPPLQDASFGNLCVVVTAVLPATTATTTNPATKKVSSTSNEEQVALDELSDFVALLRREIDKVKGDKGCMEKIIQKFIYGHDASVAKDSDVEDKVTALFMTSWCKFGFYEADFGWGTPVWVTTVPLIEPKYKNMVFMNDMKCGEGIEVWVNFLEDDMTKFEHHLREILQLF

SEQ ID NO: 21 - DNA, 350 bp, Artificial Sequence
  VIGS
tggtcataatcatcaatcagccacagtcactaaaatcactgcttctaatgaaagcagcaatggtgtctgttatctttcagaaacggctaacttggggaagttaatatgcattccaatggcactaagagctgcgatggagctaaatgtgttccaacttatctcaaagttcggaactgacgcaaaagtttcggcttctgaaattgcctctaaaatgccaaacgcgaagaataatcctgaagcagctatgtatttggatagaattcttcgactgctcggggcaagttctattctttctgtttctactacaaaaaaatcaatcaacagaggaggagatgatgtagtagtacatg

SEQ ID NO: 22 - DNA, 213 bp, artificial sequence
  VIGS
gtgtaactaagccagcgctaatacaaggatgtggcaaaatcctgaacggagttacatcgttaattgatgtcggtggtggtcacggtgccactatggcctacatagttgaagcttttcctcacataaaaggtgcggtaatcgatttaccacatgttgttgaagccgctccggagcgtccaggtgttgagttcatcagcggtgatatattcaagt

SEQ ID NO: 23 - DNA, 264 bp, artificial sequence
  VIGS
tttgagtaatggtgaaaagatggatgtggattacaaaggtcacaatcatgaattcataccatttgggataggtcggaggatgtgcgctggtatgctttgggcatcggaggtgattcatttggtgctgccccgtcttattcatgggtttgatatgaaagcagcaagtgccaatgggaaagtagatatggcagaaatggcaggcatggtgatttgttttaagaagacacctcttgaagttatggtcaatcctcgagagtagatgtt

SEQ ID NO: 24 - DNA, 119 bp, artificial sequence
  VIGS
atgatcatgagtaacttatggattcttacgctcatttctaccatattagcagtctttgctgctgtgttaatcattttcaggagaagaatatcagcatccacaacggaatggcctgttgg

SEQ ID NO: 25 - DNA, 196 bp, artificial sequence
  VIGS
taggagggtatgtccggctatagtttcatcactgcagacgatgcattatgcgttggcgcgtcttattcaaggatatgaaatgaaatcagccagcctcgatgggaaggtgaatatggaagaaatgatagccatgtcgtgccacaagatgagccctcttgaagttattatcagtcctcgggagccgaggcggagttaa

SEQ ID NO: 26 - DNA, 186 bp, artificial sequence
  VIGS
tcctatatatgctaattaattagatgaataaaatctgtggtcgagtaaatctaattaatgctaatgaacaagatgaataaaaaattttctttctgcttttgctttggttagggttatttgaccctcatttggttgtattcgttggcgcacaacttttgtgcttcttaatataattccttttggtgg

SEQ ID NO: 27 - DNA, 204 bp, artificial sequence
  VIGS
tggcagatccttatgaattcctaatgtgcattcacaatcctgaagaagataccctaacaagaaattttccgattcctgctactcccttagatcaaaacaccaaagacatttctttaaatcctgataggaaaacctcacttcgaatctttcggccaccaaccaaagaacctcctgtaacaaagaataagctgcttcctatcataa

SEQ ID NO: 28 - DNA, 323 bp, artificial sequence
  VIGS
gaaattgacgagacaatatggtcagaagttgacaatttcattagcaaaccggaacaagttattcctggattgccctcatatgtggtttcaaaggtactgacagaaagagcttgcctaaagttttctgaagaacatggtttggatgttgttactatacttcctccgttggttgttggaccttttatcactccccatcctcctcccagtgtatctatagctctttcgataatttcaggtgatgtgtcgatgatgcttggtgttagacttgaaaatgcggtacatatagatgatgttgctttagcacacatattcgtttttgaatg

SEQ ID NO: 29 - DNA, 117 bp, artificial sequence
  VIGS
cctaagagagatcctccaactgttttgattttcaaccgtttccctaatagaggtcaattgtcgtgtttgtccatcttaactaccatctttattctcttgttttcatacttgtatttg

SEQ ID NO: 30 - DNA, 129 bp, artificial sequence
  VIGS
gatcatcttctcttcagcagaagtcccctcttaagcgtatacgctgacatgtcagtgacatgcaaggaatattatgacccaaacaaatccatgcttgagttggtatttgcacccgctgaggaatggatc

SEQ ID NO: 31 - DNA, 22 bp, artificial sequence
  Primer
gattcccgatttactcctgatg

SEQ ID NO: 32 - DNA, 30 bp, artificial sequence
  Primer
aacacaaaatacgattacttacttttgtcc

SEQ ID NO: 33 - DNA, 23 bp, artificial sequence
  Primer
tgcctcatgttatttctgttgcc

SEQ ID NO: 34 - DNA, 26 bp, artificial sequence
  Primer
gcatgaaatggatgtagttatcttgg

SEQ ID NO: 35 - DNA, 22 bp, artificial sequence
  Primer
attgatgtcggtggtggtcacg

SEQ ID NO: 36 - DNA, 24 bp, artificial sequence
  Primer
attcccgttcaagtaaacatgcgg

SEQ ID NO: 37 - DNA, 27 bp, artificial sequence
  Primer
gcaactgtttcattaacaggcacatcc

SEQ ID NO: 38 - DNA, 29 bp, artificial sequence
  Primer
cagtaaattcacacattccgtatcttccc

SEQ ID NO: 39 - DNA, 24 bp, artificial sequence
  Primer
gcttcagcattggttaacgagtgc

SEQ ID NO: 40 - DNA, 26 bp, artificial sequence
  Primer
gagggtaagcctcaataacagactgg

SEQ ID NO: 41 - DNA, 23 bp, artificial sequence
  Primer
agaccgtttgtaccgaattctgc

SEQ ID NO: 42 - DNA, 22 bp, artificial sequence
  Primer
tcgttccattcgtgaagaatgc

SEQ ID NO: 43 - DNA, 25 bp, artificial sequence
  Primer
gaaccattaaacacttgagtcatgc

SEQ ID NO: 44 - DNA, 24 bp, artificial sequence
  Primer
tgcaattgaatttagctcatctcc

SEQ ID NO: 45 - DNA, 21 bp, artificial sequence
  Primer
ttgatgaacgacaaggaaccg

SEQ ID NO: 46 - DNA, 26 bp, artificial sequence
  Primer
attcatgattgtgacctttgtaatcc

SEQ ID NO: 47 - DNA, 24 bp, artificial sequence
  Primer
atgtggaaaacggtaagcaagtgg

SEQ ID NO: 48 - DNA, 25 bp, artificial sequence
  Primer
acgattctgtcatcatcattttcgc

SEQ ID NO: 49 - DNA, 23 bp, artificial sequence
  Primer
caacctcaatctagctagagtcg

SEQ ID NO: 50 - DNA, 25 bp, artificial sequence
  Primer
cccaagattttcatatcctttacaa

SEQ ID NO: 51 - DNA, 31 bp, artificial sequence
  Primer
caataattgagtaatttcagttcattcatgg

SEQ ID NO: 52 - DNA, 20 bp, artificial sequence
  Primer
gctccgtaagtgctcctgtg

SEQ ID NO: 53 - DNA, 26 bp, artificial sequence
  Primer
gaattgtggtaaaaaattagatgcag

SEQ ID NO: 54 - DNA, 22 bp, artificial sequence
  Primer
cccttcacatctaccatccctt

SEQ ID NO: 55 - DNA, 27 bp, artificial sequence
  Primer
caaagagtcaatctgactcaagctagc

SEQ ID NO: 56 - DNA, 18 bp, artificial sequence
  Primer
cgagtgcccatgcagtgg

SEQ ID NO: 57 - DNA, 28 bp, artificial sequence
  Primer
tcaaaccctgctactaacacttacttgc

SEQ ID NO: 58 - DNA, 23 bp, artificial sequence
  Primer
cactccatcagacacacaagacc

SEQ ID NO: 59 - DNA, 27 bp, artificial sequence
  Primer
ttttatcgaccttgaggaacaattagg

SEQ ID NO: 60 - DNA, 18 bp, artificial sequence
  Primer
aaatggcagttccaccgc

SEQ ID NO: 61 - DNA, 25 bp, artificial sequence
  Primer
gacttcatgatgaaatcagatgcac

SEQ ID NO: 62 - DNA, 24 bp, artificial sequence
  Primer
cactgctgacttccatatcaaagc

SEQ ID NO: 63 - DNA, 24 bp, artificial sequence
  Primer
atgctgttgatgctttaaactggg

SEQ ID NO: 64 - DNA, 26 bp, artificial sequence
  Primer
agctgaatttgtcgatcaataagtgg

SEQ ID NO: 65 - DNA, 26 bp, artificial sequence
  Primer
aataaaaatccaacaatggcagatcc

SEQ ID NO: 66 - DNA, 24 bp, artificial sequence
  Primer
actggcatgatatgcaacattagc

SEQ ID NO: 67 - DNA, 24 bp, artificial sequence
  Primer
ggaagatgtgagccaccttaaagc

SEQ ID NO: 68 - DNA, 22 bp, artificial sequence
  Primer
gatacactgggaggaggatggg

SEQ ID NO: 69 - DNA, 26 bp, artificial sequence
  Primer
gagagtaaccacatctttgttgtcgg

SEQ ID NO: 70 - DNA, 22 bp, artificial sequence
  Primer
cggcaaaattcattccttgagc

SEQ ID NO: 71 - DNA, 19 bp, artificial sequence
  Primer
gtttactcccacgtgcatc

SEQ ID NO: 72 - DNA, 23 bp, artificial sequence
  Primer
cattcctcgtctaattcatctgc

SEQ ID NO: 73 - DNA, 19 bp, artificial sequence
  Primer
gtttactcccacgtgcatc

SEQ ID NO: 74 - DNA, 24 bp, artificial sequence
  Primer
gcttcactacttcttcttgaaaag

SEQ ID NO: 75 - DNA, 18 bp, artificial sequence
  Primer
aaacaatgctggggttgc

SEQ ID NO: 76 - DNA, 26 bp, artificial sequence
  Primer
cattataatttccaatgccgtagttc

SEQ ID NO: 77 - DNA, 20 bp, artificial sequence
  Primer
taagagagggagaccacgag

SEQ ID NO: 78 - DNA, 23 bp, artificial sequence
  Primer
cattcgttgttgttgctggtaag

SEQ ID NO: 79 - DNA, 26 bp, artificial sequence
  Primer
cttatgaagctaggtaatggtatgga

SEQ ID NO: 80 - DNA, 20 bp, artificial sequence
  Primer
catcctcattgcttgtgtcc

SEQ ID NO: 81 - DNA, 19 bp, artificial sequence
  Primer
ctctaaaatgccaaacgcg

SEQ ID NO: 82 - DNA, 20 bp, artificial sequence
  Primer
gaccctttgggacttcctcg

SEQ ID NO: 83 - DNA, 19 bp, artificial sequence
  Primer
cgtgttgtttggtccctcg

SEQ ID NO: 84 - DNA, 23 bp, artificial sequence
  Primer
tgcctcatgttatttctgttgcc

SEQ ID NO: 85 - DNA, 23 bp, artificial sequence
  Primer
gattcccgatttactcctgatgg

SEQ ID NO: 86 - DNA, 30 bp, artificial sequence; identical to SEQ ID NO: 32
  Primer

SEQ ID NO: 87 - DNA, 23 bp, artificial sequence
  Primer
tgcctcatgttatttctgttgcc

SEQ ID NO: 88 - DNA, 26 bp, artificial sequence
  Primer
gcatgaaatggatgtagttatcttgg

SEQ ID NO: 89 - DNA, 21 bp, artificial sequence
  Primer
aaatcgttcgctctttaccgc

SEQ ID NO: 90 - DNA, 22 bp, artificial sequence
  Primer
cacaccaaacttgatcattgtc

SEQ ID NO: 91 - DNA, 27 bp, artificial sequence
  Primer
attgttgatattgaatcagaaactttc

SEQ ID NO: 92 - DNA, 25 bp, artificial sequence
  Primer
tcaataccagtactgttagtttccg

SEQ ID NO: 93 - DNA, 27 bp, artificial sequence
  Primer
gcaactgtttcattaacaggcacatcc

SEQ ID NO: 94 - DNA, 22 bp, artificial sequence
  Primer
attgatgtcggtggtggtcacg

SEQ ID NO: 95 - DNA, 23 bp, artificial sequence
  Primer
gcacactgtctttttcttccacc

SEQ ID NO: 96 - DNA, 28 bp, artificial sequence
  Primer
accggaatgagaatgcataaagtaaagg

SEQ ID NO: 97 - DNA, 23 bp, artificial sequence
  Primer
ccaatacccaatcaattaaactc

SEQ ID NO: 98 - DNA, 29 bp, artificial sequence
  Primer
cagtaaattcacacattccgtatcttccc

SEQ ID NO: 99 - DNA, 27 bp, artificial sequence
  Primer
attgtatagccaaagttgcaggtaggg

SEQ ID NO: 100 - DNA, 23 bp, artificial sequence
  Primer
agaccgtttgtaccgaattctgc

SEQ ID NO: 101 - DNA, 23 bp, artificial sequence
  Primer
gcagtgaaagccatatccaaagc

SEQ ID NO: 102 - DNA, 21 bp, artificial sequence
  Primer
aaccgtccccaagatgattcc

SEQ ID NO: 103 - DNA, 22 bp, artificial sequence
  Primer
tcgttccattcgtgaagaatgc

SEQ ID NO: 104 - DNA, 26 bp, artificial sequence
  Primer
gagggtaagcctcaataacagactgg

SEQ ID NO: 105 - DNA, 25 bp, artificial sequence
  Primer
gaaccattaaacacttgagtcatgc

SEQ ID NO: 106 - DNA, 21 bp, artificial sequence
  Primer
ttgatgaacgacaaggaaccg

SEQ ID NO: 107 - DNA, 19 bp, artificial sequence
  Primer
tcgacagcgcttacgaacg

SEQ ID NO: 108 - DNA, 21 bp, artificial sequence
  Primer
caattatcaaagaatcaatgc

SEQ ID NO: 109 - DNA, 22 bp, artificial sequence
  Primer
tgcaattgaatttagctcatct

SEQ ID NO: 110 - DNA, 26 bp, artificial sequence
  Primer
attcatgattgtgacctttgtaatcc

SEQ ID NO: 111 - DNA, 21 bp, artificial sequence
  Primer
gacagagggcccaagttaagg

SEQ ID NO: 112 - DNA, 20 bp, artificial sequence
  Primer
agcaaaccattcgtccatcc

SEQ ID NO: 113 - DNA, 21 bp, artificial sequence
  Primer
tacgacaggttgctagcttgg

SEQ ID NO: 114 - DNA, 24 bp, artificial sequence
  Primer
aataatggatcagtcacggcttcc

SEQ ID NO: 115 - DNA, 27 bp, artificial sequence
  Primer
aatccatcagattttcaaccagagagg

SEQ ID NO: 116 - DNA, 28 bp, artificial sequence
  Primer
tgtcagccaaccattcgtccatcctaac

SEQ ID NO: 117 - DNA, 28 bp, artificial sequence
  Primer
ggcttcccggagatgacccagattttat

SEQ ID NO: 118 - DNA, 38 bp, artificial sequence
  Primer
ttgttattttcatgactattaccaccagcttcctctta

SEQ ID NO: 119 - DNA, 30 bp, artificial sequence
  Primer
agtggaggaggcacaaaagttaggatggac

SEQ ID NO: 120 - DNA, 29 bp, artificial sequence
  Primer
ccatgtctgataaatacgggtcggtgttc

SEQ ID NO: 121 - DNA, 36 bp, artificial sequence
  Primer
ttgttgataaggacgactaagaataagcagaagata

SEQ ID NO: 122 - DNA, 25 bp, artificial sequence
  Primer
acgattctgtcatcatcattttcgc

SEQ ID NO: 123 - DNA, 24 bp, artificial sequence
  Primer
agtcgtgtatcgttcgcttaatgc

SEQ ID NO: 124 - DNA, 29 bp, artificial sequence
  Primer
catgcctatctatttcctcccttgccctc

SEQ ID NO: 125 - DNA, 28 bp, artificial sequence
  Primer
tgtcagccaaccattcgtccatcctaac

SEQ ID NO: 126 - DNA, 31 bp, artificial sequence
  Primer
tgttcgatcacgttgtctctttttgccataa

SEQ ID NO: 127 - DNA, 38 bp, artificial sequence
  Primer
taacaataaaagtactgataatggtggtcgaaggagaa

SEQ ID NO: 128 - DNA, 20 bp, artificial sequence
  Primer
tattgatgtggaccagtacc

SEQ ID NO: 129 - DNA, 20 bp, artificial sequence
  Primer
tgtaactcttggtcacatgg

SEQ ID NO: 130 - DNA, 20 bp, artificial sequence
  Primer
cgcgtacttgacatttaacg

SEQ ID NO: 131 - DNA, 20 bp, artificial sequence
  Primer
ggatcatcgccaaaagaaac

SEQ ID NO: 132 - DNA, 27 bp, artificial sequence
  Primer
caaagagtcaatctgactcaagctagc

SEQ ID NO: 133 - DNA, 26 bp, artificial sequence
  Primer
tgaaatgcctgagatcactaaaatcg

SEQ ID NO: 134 - DNA, 28 bp, artificial sequence
  Primer
tcaaaccctgctactaacacttacttgc

SEQ ID NO: 135 - DNA, 24 bp, artificial sequence
  Primer
tgtaaagacacttcattgatgggc

SEQ ID NO: 136 - DNA, 31 bp, artificial sequence
  Primer
ttcgatttgtgtaaacattaatgatatttgg

SEQ ID NO: 137 - DNA, 27 bp, artificial sequence
  Primer
gagatgatcaagtggtttaaccattcc

SEQ ID NO: 138 - DNA, 18 bp, artificial sequence
  Primer
cgagtgcccatgcagtgg

SEQ ID NO: 139 - DNA, 26 bp, artificial sequence
  Primer
aataaaaatccaacaatggcagatcc

SEQ ID NO: 140 - DNA, 24 bp, artificial sequence
  Primer
atgctgttgatgctttaaactggg

SEQ ID NO: 141 - DNA, 28 bp, artificial sequence
  Primer
ggttaatcgagagatgttttgtggtagg

SEQ ID NO: 142 - DNA, 23 bp, artificial sequence
  Primer
cgatgacacagagcaagaacgac

SEQ ID NO: 143 - DNA, 23 bp, artificial sequence
  Primer
cgcgggtatatgtgtagcaatcg

SEQ ID NO: 144 - DNA, 17 bp, artificial sequence
  Primer
cggcaacgccagttccc

SEQ ID NO: 145 - DNA, 26 bp, artificial sequence
  Primer
ctaacaggcaaacaataacaggttgc

SEQ ID NO: 146 - DNA, 24 bp, artificial sequence
  Primer
ggaagatgtgagccaccttaaagc

SEQ ID NO: 147 - DNA, 26 bp, artificial sequence
  Primer
aaaggtactgacagaaagagcttgcc

SEQ ID NO: 148 - DNA, 23 bp, artificial sequence
  Primer
agatacactgggaggaggatggg

SEQ ID NO: 149 - DNA, 22 bp, artificial sequence
  Primer
cggcaaaattcattccttgagc

SEQ ID NO: 150 - DNA, 24 bp, artificial sequence
  Primer
aacatatagccaaaggactcttcg

SEQ ID NO: 151 - DNA, 20 bp, artificial sequence
  Primer
aggatacacaatgacccaac

SEQ ID NO: 152 - DNA, 27 bp, artificial sequence
  Primer
ttttatcgaccttgaggaacaattagg

SEQ ID NO: 153 - DNA, 20 bp, artificial sequence
  Primer
tgttcactaggtggaaagag

SEQ ID NO: 154 - DNA, 26 bp, artificial sequence
  Primer
agtacaataccgagaaatccgacaag

SEQ ID NO: 155 - DNA, 27 bp, artificial sequence
  Primer
gctcaattaatggaacagtagttaccc

SEQ ID NO: 156 - DNA, 19 bp, artificial sequence
  Primer
cgtgttgtttggtccctcg

SEQ ID NO: 157 - DNA, 23 bp, Artificial Sequence
  Primer
gcacactgtctttttcttccacc

SEQ ID NO: 158 - DNA, 27 bp, Artificial Sequence
  Primer
gcaactgtttcattaacaggcacatcc

SEQ ID NO: 159 - DNA, 24 bp, artificial sequence
  Primer
gccagcgctaatacaaggatgtgg

SEQ ID NO: 160 - DNA, 23 bp, artificial sequence
  Primer
gcagtgaaagccatatccaaagc

SEQ ID NO: 161 - DNA, 22 bp, artificial sequence
  Primer
tcgttccattcgtgaagaatgc

SEQ ID NO: 162 - DNA, 23 bp, artificial sequence
  Primer
gctacgaaagataatggtgcagc

SEQ ID NO: 163 - DNA, 20 bp, artificial sequence
  Primer
agcaaaccattcgtccatcc

SEQ ID NO: 164 - DNA, 24 bp, artificial sequence
  Primer
atgtggaaaacggtaagcaagtgg

SEQ ID NO: 165 - DNA, 25 bp, artificial sequence
  Primer
acgattctgtcatcatcattttcgc

SEQ ID NO: 166 - DNA, 26 bp, artificial sequence
  Primer
tgaaatgcctgagatcactaaaatcg

SEQ ID NO: 167 - DNA, 27 bp, artificial sequence
  Primer
ggaatggttaaaccacttgatcatctc

SEQ ID NO: 168 - DNA, 27 bp, artificial sequence
  Primer
atgccagtttaagagcaatagaaatgg

SEQ ID NO: 169 - DNA, 17 bp, artificial sequence
  Primer
gggaactggcgttgccg

SEQ ID NO: 170 - DNA, 23 bp, artificial sequence
  Primer
gaagatgtgagccaccttaaagc

SEQ ID NO: 171 - DNA, 22 bp, artificial sequence
  Primer
gctcaaggaatgaattttgccg

SEQ ID NO: 172 - DNA, 21 bp, artificial sequence
  Primer
gttgacgcaggaagcttttgc

SEQ ID NO: 173 - DNA, 25 bp, artificial sequence
  Primer
ggaacataagatttaactccgcctc

SEQ ID NO: 174 - DNA, 34 bp, artificial sequence
  Primer
aaactcgagaagcttggtcataatcatcaatcag

SEQ ID NO: 175 - DNA, 31 bp, artificial sequence
  Primer
aaaggtacccatgtactactacatcatctcc

SEQ ID NO: 176 - DNA, 33 bp, artificial sequence
  Primer
aaactcgagaagcttgtgtaactaagccagcgc

SEQ ID NO: 177 - DNA, 27 bp, artificial sequence
  Primer
aaaggtaccacttgaatatatcaccgc

SEQ ID NO: 178 - DNA, 29 bp, artificial sequence
  Primer
aaaggatcctttgagtaatggtgaaaaga

SEQ ID NO: 179 - DNA, 30 bp, artificial sequence
  Primer
aaaggtaccaacatctactctcgaggattg

SEQ ID NO: 180 - DNA, 33 bp, artificial sequence
  Primer
aaactcgagaagctttaggagggtatgtccggc

SEQ ID NO: 181 - DNA, 28 bp, artificial sequence
  Primer
aaaggtaccttaactccgcctcggctcc

SEQ ID NO: 182 - DNA, 27 bp, artificial sequence
  Primer
aaaggatccttcagttcattcatggcg

SEQ ID NO: 183 - DNA, 33 bp, artificial sequence
  Primer
aaaggtaccgttcatagtaaataataacaggcg

SEQ ID NO: 184 - DNA, 37 bp, artificial sequence
  Primer
aaactcgagaagcttatgatcatgagtaacttatgga

SEQ ID NO: 185 - DNA, 28 bp, artificial sequence
  Primer
aaaggtaccccaacaggccattccgttg

SEQ ID NO: 186 - DNA, 30 bp, artificial sequence
  Primer
aaaggatcctggcagatccttatgaattcc

SEQ ID NO: 187 - DNA, 32 bp, artificial sequence
  Primer
aaaggtaccttatgataggaagcagcttattc

SEQ ID NO: 188 - DNA, 30 bp, artificial sequence
  Primer
aaaggatccgaaattgacgagacaatatgg

SEQ ID NO: 189 - DNA, 32 bp, artificial sequence
  Primer
aaaggtacccattcaaaaacgaatatgtgtgc

SEQ ID NO: 190 - DNA, 31 bp, artificial sequence
  Primer
aaaggatcccctaagagagatcctccaactg

SEQ ID NO: 191 - DNA, 36 bp, artificial sequence
  Primer
aaaggtaccaatacaagtatgaaaacaagagaataa

SEQ ID NO: 192 - DNA, 22 bp, artificial sequence
  Primer
gaggtgttcattgccatgtcaa

SEQ ID NO: 193 - DNA, 22 bp, artificial sequence
  Primer
gtttcgcaagctcctgcatagt

SEQ ID NO: 194 - DNA, 39 bp, Artificial Sequence
  Primer
  misc_feature (12)..(12): R = A or G;
  misc_feature (38)..(38): V = A,  C or G
  misc_feature (39)..(39): N = A/T or C/G
attctagatccracatgttttttttttttttttttttvn